European Patent Application EP 4 233 843 A2, published August 30, 2023. Title: ANTIBODY COMPOSITIONS. Applicant: PHILOGEN S.P.A. Application EP. The sequence listing filed with the application follows.

SEQUENCE LISTING (8 sequences)

SEQ ID NO: 1 - protein, 410 aa, synthetic construct
  REGION 1..410: note = L19-TNFalpha
EVQLLESGGGLVQPGGSLRLSCAASGFTFSSFSMSWVRQAPGKGLEWVSSISGSSGTTYYADSVKGRFTISRDNSKNTLYLQMNSLRAEDTAVYYCAKPFPYFDYWGQGTLVTVSSGDGSSGGSGGASEIVLTQSPGTLSLSPGERATLSCRASQSVSSSFLAWYQQKPGQAPRLLIYYASSRATGIPDRFSGSGSGTDFTLTISRLEPEDFAVYYCQQTGRIPPTFGQGTKVEIKEFSSSSGSSSSGSSSSGVRSSSRTPSDKPVAHVVANPQAEGQLQWLNRRANALLANGVELRDNQLVVPSEGLYLIYSQVLFKGQGCPSTHVLLTHTISRIAVSYQTKVNLLSAIKSPCQRETPEGAEAKPWYEPIYLGGVFQLEKGDRLSAEINRPDYLDFAESGQVYFGIIAL

SEQ ID NO: 2 - protein, 386 aa, synthetic construct
  REGION 1..386: note = L19-IL2
EVQLLESGGGLVQPGGSLRLSCAASGFTFSSFSMSWVRQAPGKGLEWVSSISGSSGTTYYADSVKGRFTISRDNSKNTLYLQMNSLRAEDTAVYYCAKPFPYFDYWGQGTLVTVSSGDGSSGGSGGASEIVLTQSPGTLSLSPGERATLSCRASQSVSSSFLAWYQQKPGQAPRLLIYYASSRATGIPDRFSGSGSGTDFTLTISRLEPEDFAVYYCQQTGRIPPTFGQGTKVEIKEFSSSSGSSSSGSSSSGAPTSSSTKKTQLQLEHLLLDLQMILNGINNYKNPKLTRMLTFKFYMPKKATELKHLQCLEEELKPLEEVLNLAQSKNFHLRPRDLISNINVIVLELKGSETTFMCEYADETATIVEFLNRWITFCQSIISTLT

SEQ ID NO: 3 - protein, 116 aa, synthetic construct [sequence omitted]

SEQ ID NO: 4 - protein, 12 aa, synthetic construct
  REGION 1..12: note = scFV Linker
GDGSSGGSGGAS

SEQ ID NO: 5 - protein, 108 aa, synthetic construct [sequence omitted]

SEQ ID NO: 6 - protein, 17 aa, synthetic construct
  REGION 1..17: note = Linker
EFSSSSGSSSSGSSSSG

SEQ ID NO: 7 - protein, 157 aa, synthetic construct [sequence omitted]

SEQ ID NO: 8 - protein, 133 aa, synthetic construct [sequence omitted]